European Patent Application EP 4 696 707 A1, published February 18, 2026. Title: SINGLE FUSION PROTEIN AND PHARMACEUTICAL COMPOSITION COMPRISING SAME. Applicant: MEDI&GENE. The sequence listing filed with the application follows.

SEQUENCE LISTING (46 sequences)

SEQ ID NO: 1 - protein, 297 aa, Artificial Sequence
GSDQSENVDRGAGSIREAGGAFGKREQAEEERYFRAQSREQLAALKKHHEEEIVHHKKEIGGGGSEPKSCDKTHTCPPCPAPEAAGGPSVFLFPPKPKDTLMISRTPEVTCVVVDVSHEDPEVKFNWYVDGVEVHNAKTKPREEQYNSTYRVVSVLTVLHQDWLNGKEYKCKVSNKALPAPIEKTISKAKGQPREPQVYTLPPSRDELTKNQVSLTCLVKGFYPSDIAVEWESNGQPENNYKTTPPVLDSDGSFFLYSKLTVDKSRWQQGNVFSCSVMHEALHNHYTQKSLSLSPGK

SEQ ID NO: 2 - protein, 307 aa, Artificial Sequence
GSDQSENVDRGAGSIREAGGAFGKREQAEEERYFRAQSREQLAALKKHHEEEIVHHKKEIGGGGSGGGGSGGGGSEPKSCDKTHTCPPCPAPEAAGGPSVFLFPPKPKDTLMISRTPEVTCVVVDVSHEDPEVKFNWYVDGVEVHNAKTKPREEQYNSTYRVVSVLTVLHQDWLNGKEYKCKVSNKALPAPIEKTISKAKGQPREPQVYTLPPSRDELTKNQVSLTCLVKGFYPSDIAVEWESNGQPENNYKTTPPVLDSDGSFFLYSKLTVDKSRWQQGNVFSCSVMHEALHNHYTQKSLSLSPGK

SEQ ID NO: 3 - protein, 307 aa, Artificial Sequence
GSDQSENVDRGAGSIREAGSAFGKREQAEEERYMRAQSREQLAALKKHHEEEIVHHKKEIGGGGSGGGGSGGGGSEPKSCDKTHTCPPCPAPEAAGGPSVFLFPPKPKDTLMISRTPEVTCVVVDVSHEDPEVKFNWYVDGVEVHNAKTKPREEQYNSTYRVVSVLTVLHQDWLNGKEYKCKVSNKALPAPIEKTISKAKGQPREPQVYTLPPSRDELTKNQVSLTCLVKGFYPSDIAVEWESNGQPENNYKTTPPVLDSDGSFFLYSKLTVDKSRWQQGNVFSCSVMHEALHNHYTQKSLSLSPGK

SEQ ID NO: 4 - protein, 306 aa, Artificial Sequence
SPILGYWKIKGLVQPTRLLLEYLEEKYEEHLYERDEGDKWRNKKFELGLEFPNLPYYIDGDVKLTQSMAIIRYIADKHNMLGGCPKERAEISMLEGAVLDIRYGVSRIAYSKDFETLKVDFLSKLPEMLKMFEDRLCHKTYLNGDHVTHPDFMLYDALDVVLYMDPMCLDAFPKLVCFKKRIEAIPQIDKYLKSSKYIAWPLQGWQATFGGGDHPPKSDLVPRGSGSDQSENVDRGAGSIREAGGAFGKREQAEEERYFRAQSREQLAALKKHHEEEIVHHKKEIERLQKEIERHKQKIKMLKHDD

SEQ ID NO: 5 - protein, 101 aa, Artificial Sequence
MGSHHHHHHSSGLVPRGSHMGSDQSENVDRGAGSIREAGGAFGKREQAEEERYFRAQSREQLAALKKHHEEEIVHHKKEIERLQKEIERHKQKIKMLKHDD

SEQ ID NO: 6 - protein, 285 aa, Artificial Sequence
SPILGYWKIKGLVQPTRLLLEYLEEKYEEHLYERDEGDKWRNKKFELGLEFPNLPYYIDGDVKLTQSMAIIRYIADKHNMLGGCPKERAEISMLEGAVLDIRYGVSRIAYSKDFETLKVDFLSKLPEMLKMFEDRLCHKTYLNGDHVTHPDFMLYDALDVVLYMDPMCLDAFPKLVCFKKRIEAIPQIDKYLKSSKYIAWPLQGWQATFGGGDHPPKSDLVPRGSGSDQSENVDRGAGSIREAGGAFGKREQAEEERYFRAQSREQLAALKKHHEEEIVHHKKEI

SEQ ID NO: 7 - protein, 351 aa, Artificial Sequence
GSDQSENVDRGAGSIREAGGAFGKREQAEEERYFRAQSREQLAALKKHHEEEIVHHKKEIGGGGSGGGGSGGGGSHGEGTFTSDVSSYLEEQAAKEFIAWLVKGGGGGGGSGGGGSGGGGSAESKYGPPCPPCPAPEFLGGPSVFLFPPKPKDTLMISRTPEVTCVVVDVSQEDPEVQFNWYVDGVEVHNAKTKPREEQFNSTYRVVSVLTVLHQDWLNGKEYKCKVSNKGLPSSIEKTISKAKGQPREPQVYTLPPSQEEMTKNQVSLTCLVKGFYPSDIAVEWESNGQPENNYKTTPPVLDSDGSFFLYSRLTVDKSRWQEGNVFSCSVMHEALHNHYTQKSLSLSLGK

SEQ ID NO: 8 - protein, 81 aa, Homo sapiens
GSDQSENVDRGAGSIREAGGAFGKREQAEEERYFRAQSREQLAALKKHHEEEIVHHKKEIERLQKEIERHKQKIKMLKHDD

SEQ ID NO: 9 - protein, 60 aa, Homo sapiens
GSDQSENVDRGAGSIREAGGAFGKREQAEEERYFRAQSREQLAALKKHHEEEIVHHKKEI

SEQ ID NO: 10 - protein, 47 aa, Homo sapiens
GSDQSENVDRGAGSIREAGGAFGKREQAEEERYFRAQSREQLAALKK

SEQ ID NO: 11 - protein, 40 aa, Artificial Sequence
RGAGSIREAGGAFGKREQAEEERYFRAQSREQLAALKKHK

SEQ ID NO: 12 - protein, 28 aa, Homo sapiens
VDRGAGSIREAGGAFGKREQAEEERYFR

SEQ ID NO: 13 - protein, 317 aa, Artificial Sequence
GSDQSENVDRGAGSIREAGGAFGKREQAEEERYFRAQSREQLAALKKHHEEEIVHHKKEIERLQKEIERHKQKIKMLKHDDGGGGSEPKSQDKTHTCPPCPAPELLGGPSVFLFPPKPKDTLMISRTPEVTCVVVDVSHEDPEVKFNWYVDGVEVHNAKTKPREEQYNSTYRVVSVLTVLHQDWLNGKEYKCKVSNKALPAPIEKTISKAKGQPREPQVYTLPPSRDELTKNQVSLTCLVKGFYPSDIAVEWESNGQPENNYKTTPPVLDSDGSFFLYSKLTVDKSRWQQGNVFSCSVMHEALHNHYTQKSLSLSPG

SEQ ID NO: 14 - protein, 296 aa, Artificial Sequence
GSDQSENVDRGAGSIREAGGAFGKREQAEEERYFRAQSREQLAALKKHHEEEIVHHKKEIGGGGSEPKSQDKTHTCPPCPAPELLGGPSVFLFPPKPKDTLMISRTPEVTCVVVDVSHEDPEVKFNWYVDGVEVHNAKTKPREEQYNSTYRVVSVLTVLHQDWLNGKEYKCKVSNKALPAPIEKTISKAKGQPREPQVYTLPPSRDELTKNQVSLTCLVKGFYPSDIAVEWESNGQPENNYKTTPPVLDSDGSFFLYSKLTVDKSRWQQGNVFSCSVMHEALHNHYTQKSLSLSPG

SEQ ID NO: 15 - protein, 283 aa, Artificial Sequence
GSDQSENVDRGAGSIREAGGAFGKREQAEEERYFRAQSREQLAALKKGGGGSEPKSQDKTHTCPPCPAPELLGGPSVFLFPPKPKDTLMISRTPEVTCVVVDVSHEDPEVKFNWYVDGVEVHNAKTKPREEQYNSTYRVVSVLTVLHQDWLNGKEYKCKVSNKALPAPIEKTISKAKGQPREPQVYTLPPSRDELTKNQVSLTCLVKGFYPSDIAVEWESNGQPENNYKTTPPVLDSDGSFFLYSKLTVDKSRWQQGNVFSCSVMHEALHNHYTQKSLSLSPG

SEQ ID NO: 16 - protein, 28 aa, Artificial Sequence
ADRGAGSIREAGGAFGKREQAEEERYFR

SEQ ID NO: 17 - protein, 28 aa, Artificial Sequence
VARGAGSIREAGGAFGKREQAEEERYFR

SEQ ID NO: 18 - protein, 28 aa, Artificial Sequence
VDAGAGSIREAGGAFGKREQAEEERYFR

SEQ ID NO: 19 - protein, 28 aa, Artificial Sequence
VDRAAGSIREAGGAFGKREQAEEERYFR

SEQ ID NO: 20 - protein, 28 aa, Artificial Sequence
VDRGAASIREAGGAFGKREQAEEERYFR

SEQ ID NO: 21 - protein, 28 aa, Artificial Sequence
VDRGAGAIREAGGAFGKREQAEEERYFR

SEQ ID NO: 22 - protein, 28 aa, Artificial Sequence
VDRGAGSAREAGGAFGKREQAEEERYFR

SEQ ID NO: 23 - protein, 28 aa, Artificial Sequence
VDRGAGSIAEAGGAFGKREQAEEERYFR

SEQ ID NO: 24 - protein, 28 aa, Artificial Sequence
VDRGAGSIRAAGGAFGKREQAEEERYFR

SEQ ID NO: 25 - protein, 28 aa, Artificial Sequence
VDRGAGSIREAAGAFGKREQAEEERYFR

SEQ ID NO: 26 - protein, 28 aa, Artificial Sequence
VDRGAGSIREAGAAFGKREQAEEERYFR

SEQ ID NO: 27 - protein, 28 aa, Artificial Sequence
VDRGAGSIREAGGAAGKREQAEEERYFR

SEQ ID NO: 28 - protein, 28 aa, Artificial Sequence
VDRGAGSIREAGGAFAKREQAEEERYFR

SEQ ID NO: 29 - protein, 28 aa, Artificial Sequence
VDRGAGSIREAGGAFGAREQAEEERYFR

SEQ ID NO: 30 - protein, 28 aa, Artificial Sequence
VDRGAGSIREAGGAFGKAEQAEEERYFR

SEQ ID NO: 31 - protein, 28 aa, Artificial Sequence
VDRGAGSIREAGGAFGKRAQAEEERYFR

SEQ ID NO: 32 - protein, 28 aa, Artificial Sequence
VDRGAGSIREAGGAFGKREAAEEERYFR

SEQ ID NO: 33 - protein, 28 aa, Artificial Sequence
VDRGAGSIREAGGAFGKREQAAEERYFR

SEQ ID NO: 34 - protein, 28 aa, Artificial Sequence
VDRGAGSIREAGGAFGKREQAEAERYFR

SEQ ID NO: 35 - protein, 28 aa, Artificial Sequence
VDRGAGSIREAGGAFGKREQAEEARYFR

SEQ ID NO: 36 - protein, 28 aa, Artificial Sequence
VDRGAGSIREAGGAFGKREQAEEEAYFR

SEQ ID NO: 37 - protein, 28 aa, Artificial Sequence
VDRGAGSIREAGGAFGKREQAEEERAFR

SEQ ID NO: 38 - protein, 28 aa, Artificial Sequence
VDRGAGSIREAGGAFGKREQAEEERYAR

SEQ ID NO: 39 - protein, 28 aa, Artificial Sequence
VDRGAGSIREAGGAFGKREQAEEERYFA

SEQ ID NO: 40 - protein, 5 aa, Artificial Sequence
GGGGS

SEQ ID NO: 41 - protein, 15 aa, Artificial Sequence
GGGGSGGGGSGGGGS

SEQ ID NO: 42 - protein, 232 aa, Artificial Sequence
EPKSCDKTHTCPPCPAPEAAGGPSVFLFPPKPKDTLMISRTPEVTCVVVDVSHEDPEVKFNWYVDGVEVHNAKTKPREEQYNSTYRVVSVLTVLHQDWLNGKEYKCKVSNKALPAPIEKTISKAKGQPREPQVYTLPPSRDELTKNQVSLTCLVKGFYPSDIAVEWESNGQPENNYKTTPPVLDSDGSFFLYSKLTVDKSRWQQGNVFSCSVMHEALHNHYTQKSLSLSPGK

SEQ ID NO: 43 - protein, 229 aa, Artificial Sequence
ESKYGPPCPPCPAPEFLGGPSVFLFPPKPKDTLMISRTPEVTCVVVDVSQEDPEVQFNWYVDGVEVHNAKTKPREEQFNSTYRVVSVLTVLHQDWLNGKEYKCKVSNKGLPSSIEKTISKAKGQPREPQVYTLPPSQEEMTKNQVSLTCLVKGFYPSDIAVEWESNGQPENNYKTTPPVLDSDGSFFLYSRLTVDKSRWQEGNVFSCSVMHEALHNHYTQKSLSLSLGK

SEQ ID NO: 44 - protein, 31 aa, Artificial Sequence
HGEGTFTSDVSSYLEEQAAKEFIAWLVKGGG

SEQ ID NO: 45 - protein, 16 aa, Artificial Sequence
GGGGSGGGGSGGGGSA

SEQ ID NO: 46 - protein, 60 aa, Artificial Sequence
GSDQSENVDRGAGSIREAGSAFGKREQAEEERYMRAQSREQLAALKKHHEEEIVHHKKEI